European Patent Application EP 4 610 360 A1, published September 3, 2025. Title: Method for producing recombinant protein using PDI derived from Trichoderma sp. strain. Applicant: CJ CheilJedang Corporation. Application KR. The sequence listing filed with the application follows.

SEQUENCE LISTING (31 sequences)

SEQ ID NO: 1 - DNA, 1595 bp, synthetic construct
  misc_feature 1..1595: note = DNA template comprising FRT region, restriction enzyme recogition site, LRA3, Flp recombinant enzyme
  source 1..1595: mol_type = other DNA
gaagttcctatactttctagagaataggaacttcactcactcagatctatcatcggtacctctatcatctgcggccgcgaagttcctatactttctagagaataggaacttccaactgacagaatgactgactccctacaccttcttcgtacagtcttacataattcggaaaaaagatatcgcgagaaacctccatacggatgatagttagcccgttcccaccacttcggctgattgttaggttacgtggggttgaaagatggagactataaagcctgatccaaagaaggccatttaccccagaatttttatctcctaaaaatatgccacaatttgatatattatgtaaaacaccacctaaggtgcttgttcgtcagtttgtggaaaggtttgaaagaccttcaggtgagaaaatagcattatgtgctgctgaactaacctatttatgttggatgattacacataacggaacagcaatcaagagagccacattcatgagctataatactatcataagcaattcgctgagtttcgatattgtcaataaatcactccagtttaaatacaagacgcaaaaagcaacaattctggaagcctcattaaagaaattgattcctgcttgggaatttacaattattccttactatggacaaaaacatcaatctgatatcactgatattgtaagtagtttgcaattacagttcgaatcatcggaggaagcagataagggaaatagccacagtaaaaaaatgcttaaagcacttctaagtgagggtgaaagcatctgggagatcactgagaaaatactaaattcgtttgagtatacttcgagatttacaaaaacaaaaactttataccaattcctcttcctagctactttcatcaattgtggaagattcagcgatattaagaacgttgatccgaaatcatttaaattagtccaaaataagtatctgggagtaataatccagtgtttagtgacagagacaaagacaagcgttagtaggcacatatacttctttagcgcaaggggtaggatcgatccacttgtatatttggatgaatttttgaggaattctgaaccagtcctaaaacgagtaaataggaccggcaattcttcaagcaataaacaggaataccaattattaaaagataacttagtcagatcgtacaataaagctttgaagaaaaatgcgccttattcaatctttgctataaaaaatggcccaaaatctcacattggaagacatttgatgacctcatttctttcaatgaagggcctaacggagttgactaatgttgtgggaaattggagcgataagcgtgcttctgccgtggccaggacaacgtatactcatcagataacagcaatacctgatcactacttcgcactagtttctcggtactatgcatatgatccaatatcaaaggaaatgatagcattgaaggatgagactaatccaattgaggagtggcagcatatagaacagctaaagggtagtgctgaaggaagcatacgataccccgcatggaatgggataatatcacaggaggtactagactacctttcatcctacataaatagacgcatataa

SEQ ID NO: 2 - DNA, 20 bp, synthetic construct
  misc_feature 1..20: note = primer 1
  source 1..20: mol_type = other DNA
gaagttcctatactttctag

SEQ ID NO: 3 - DNA, 20 bp, synthetic construct
  misc_feature 1..20: note = primer 2
  source 1..20: mol_type = other DNA
ttatatgcgtctatttatgt

SEQ ID NO: 4 - DNA, 40 bp, synthetic construct
  misc_feature 1..40: note = primer 3
  source 1..40: mol_type = other DNA
acataaatagacgcatataagtttgtagccttagacatga

SEQ ID NO: 5 - DNA, 40 bp, synthetic construct
  misc_feature 1..40: note = primer 4
  source 1..40: mol_type = other DNA
ctagaaagtataggaacttcgatctcatgaccaaaatccc

SEQ ID NO: 6 - protein, 685 aa, synthetic construct
  REGION 1..685: note = Bovine Transferrin_N495Q_amino acid sequence
DPERTVRWCTISTHEANKCASFRENVLRILESGPFVSCVKKTSHMDCIKAISNNEADAVTLDGGLVYEAGLKPNNLKPVVAEFHGTKDNPQTHYYAVAVVKKDTDFKLNELRGKKSCHTGLGRSAGWNIPMGKLYKELPDPQESIQRAAANFFSASCVPCADQSSFPKLCQLCAGKGTDKCACSNHEPYFGYSGAFKCLMEGAGDVAFVKHSTVFDNLPNPEDRKNYELLCGDNTRKSVDDYQECYLAMVPSHAVVARTVGGKEDVIWELLNHAQEHFGKDKPDNFQLFQSPHGKDLLFKDSADGFLKIPSKMDFELYLGYEYVTALQNLRESKPPDSSKDECMVKWCAIGHQERTKCDRWSGFSGGAIECETAENTEECIAKIMKGEADAMSLDGGYLYIAGKCGLVPVLAENYKTEGESCKNTPEKGYLAVAVVKTSDANINWNNLKDKKSCHTAVDRTAGWNIPMGLLYSKINNCKFDEFFSAGCAPGSPRQSSLCALCIGSEKGTGKECVPNSNERYYGYTGAFRCLVEKGDVAFVKDQTVIQNTDGNNNEAWAKNLKKENFEVLCKDGTRKPVTDAENCHLARGPNHAVVSRKDKATCVEKILNKQQDDFGKSVTDCTSNFCLFQSNSKDLLFRDDTKCLASIAKKTYDSYLGDDYVRAMTNLRQCSTSKLLEACTFHKP

SEQ ID NO: 7 - DNA, 2058 bp, synthetic construct
  misc_feature 1..2058: note = Bovine Transferrin_N495Q_nt sequence
  source 1..2058: mol_type = other DNA
gacccagaacgtacggttaggtggtgcactatatcaacacacgaggctaataaatgtgcttcttttagggagaatgtcctacgtatcctggagtctggcccattcgtctcttgcgttaaaaagacctcccacatggactgcattaaagccatctctaataatgaggccgatgcagtgaccttggatggcggtcttgtatatgaagctggtttgaaacccaataatctgaagccagttgttgcagagttccatggaaccaaggataacccacaaacccattattacgccgtggctgttgtaaaaaaggatacagattttaagttgaatgaacttagaggcaagaagtcatgtcatacgggtcttggaagatccgctggctggaacattccaatgggcaagttatacaaagagttacccgacccacaagaatctatccaaagggcagctgcaaacttttttagtgcctcttgcgtaccttgcgcagatcaatccagtttccccaagttgtgccagctatgcgcaggcaagggtactgacaaatgcgcatgctctaaccatgagccatattttggttatagtggtgctttcaagtgtttgatggaaggagcaggcgatgttgcctttgtaaagcattcaactgtcttcgacaacttgccaaatcccgaggacaggaaaaactacgaactgttgtgtggtgacaatacacgtaaatctgtagatgactaccaagagtgttacctggccatggtcccttctcacgccgttgtggcaagaactgttggtggtaaagaggatgttatctgggagttgttgaaccatgctcaagagcatttcggaaaggataaacccgataattttcaacttttccagagtccccacggcaaagatctgcttttcaaggactccgcagacggttttttgaagattccttccaaaatggatttcgagctttacttgggctatgaatatgtaaccgcccttcaaaacctgagggagtctaagcctcccgactcttctaaagacgagtgtatggtcaaatggtgcgctatcggtcatcaagagcgtacaaaatgcgataggtggagtggtttcagtggaggcgccatagagtgcgaaactgctgaaaatacggaggaatgcatcgccaaaattatgaaaggagaagcagacgctatgtctttagatggcggctatttatatatagcaggtaagtgcggcttggttcccgtactagctgagaattacaaaactgaaggcgaatcctgtaaaaacacgcccgaaaaaggttacctagctgttgccgtggtgaaaacctccgacgccaacataaattggaataacttaaaagataaaaaatcatgtcacaccgctgtagataggacagctggttggaatataccaatgggtctgttatattcaaagataaacaattgcaagtttgatgagttcttctctgctggatgtgcaccaggatcaccacgtcagtcttctttgtgtgcactgtgtattggtagtgaaaagggaaccggaaaagagtgcgtccctaattccaacgaaaggtactatggttatactggcgcctttaggtgcttggtggaaaagggagatgtggccttcgttaaggaccagaccgtcattcaaaatactgacggcaataataacgaggcatgggctaagaaccttaaaaaagagaactttgaagtcttgtgtaaggacggaaccaggaagccagtaacagatgcagaaaactgtcacttagcaagaggacctaatcatgccgtagtgtctagaaaggacaaggcaacatgcgtggagaagattttaaataagcagcaagacgattttggaaaatcagttactgattgcacatccaacttctgtctgttccagtctaacagtaaagatttgttatttagggacgatacaaaatgtctagcctcaatcgccaagaagacatacgactcatacttgggtgatgactacgtgcgtgctatgacaaatctaaggcaatgttcaacgtcaaaactattagaagcctgtactttccataaaccataa

SEQ ID NO: 8 - DNA, 40 bp, synthetic construct
  misc_feature 1..40: note = primer 5
  source 1..40: mol_type = other DNA
ctcagatctatcatcggtacagatctaacatccaaagacg

SEQ ID NO: 9 - DNA, 40 bp, synthetic construct
  misc_feature 1..40: note = primer 6
  source 1..40: mol_type = other DNA
agaaagtataggaacttcgcagcaacgttgtcactgaagt

SEQ ID NO: 10 - DNA, 18 bp, synthetic construct
  misc_feature 1..18: note = primer 7
  source 1..18: mol_type = other DNA
cgcagatcgggaacactg

SEQ ID NO: 11 - DNA, 18 bp, synthetic construct
  misc_feature 1..18: note = primer 8
  source 1..18: mol_type = other DNA
cgcagatcgggaacactg

SEQ ID NO: 12 - protein, 517 aa, synthetic construct
  REGION 1..517: note = Pichia pastoris PDI_amino acid sequence
MQFNWNIKTVASILSALTLAQASDQEAIAPEDSHVVKLTEATFESFITSNPHVLAEFFAPWCGHCKKLGPELVSAAEILKDNEQVKIAQIDCTEEKELCQGYEIKGYPTLKVFHGEVEVPSDYQGQRQSQSIVSYMLKQSLPPVSEINATKDLDDTIAEAKEPVIVQVLPEDASNLESNTTFYGVAGTLREKFTFVSTKSTDYAKKYTSDSTPAYLLVRPGEEPSVYSGEELDETHLVHWIDIESKPLFGDIDGSTFKSYAEANIPLAYYFYENEEQRAAAADIIKPFAKEQRGKINFVGLDAVKFGKHAKNLNMDEEKLPLFVIHDLVSNKKFGVPQDQELTNKDVTELIEKFIAGEAEPIVKSEPIPEIQEEKVFKLVGKAHDEVVFDESKDVLVKYYAPWCGHCKRMAPAYEELATLYANDEDASSKVVIAKLDHTLNDVDNVDIQGYPTLILYPAGDKSNPQLYDGSRDLESLAEFVKERGTHKVDALALRPVEEEKEAEEEAESEADAHDEL

SEQ ID NO: 13 - protein, 515 aa, synthetic construct
  REGION 1..515: note = Ogataea angusta PDI_amino acid sequence
MKLFNVSILTSVLAVMAVARGDADEAAIASPDSAVVKLTAESFESFIKENPLVLAEFFAPWCGHCKRLGPEFSAAADKLVEKDIKLAQIDCTQERDLCADYGIRGYPSLKVFRGNNSPSDYQGQREQDAIVSYMIKQALPPVSLLEDTADLLDALAELSEPMILQVLPPDSKSSGNETFHSLANRLRDEFRFVSTSNPEYVEKYVKEKSTPTYVVFRPGEKTEDASVLTNKTIDEEGLEKFISVETKPLFGEVTGATFQSYMDSKIPLAYFFYEEESQKAAVADEITKLAKKYRGEINFAGLEAKKYGLHAKNLNMQEKFPLFAIHDLQGDLKYGISQDKDLDFSEIPKFVENFKKGKLEPIVKSEPIPETQEEAVYHLVGYEHDKIVNQEKDVLVEYYAPWCGHCKRLAPTYEELAAIYKNDTAASAKVLIAKIDHTANDVSGVEITGYPTIFLYPADGSGPVNYEGQRTLESLASFIQEKGTFGVDGLAIRDAKSAGADGPESDAKDSTHDEL

SEQ ID NO: 14 - protein, 502 aa, synthetic construct
  REGION 1..502: note = Trichoderma reesei PDI_amino acid sequence
MQQKRLTAALVAALAAVVSAESDVKSLTKDTFNDFINSNDLVLAEFFAPWCGHCKALAPEYEEAATTLKDKSIKLAKVDCVEEADLCKEHGVEGYPTLKVFRGLDKVAPYTGPRKADGITSYMVKQSLPAVSALTKDTLEDFKTADKVVLVAYIAADDKASNETFTALANELRDTYLFGGVNDAAVAEAEGVKFPSIVLYKSFDEGKNVFSEKFDAEAIRNFAQVAATPLVGEVGPETYAGYMSAGIPLAYIFAETAEERENLAKTLKPVAEKYKGKINFATIDAKNFGSHAGNINLKTDKFPAFAIHDIEKNLKFPFDQSKEITEKDIAAFVDGFSSGKIEASIKSEPIPETQEGPVTVVVAHSYKDIVLDDKKDVLIEFYAPWCGHCKALAPKYDELASLYAKSDFKDKVVIAKVDATANDVPDEIQGFPTIKLYPAGDKKNPVTYSGARTVEDFIEFIKENGKYKAGVEIPAEPTEEAEASESKASEEAKASEETHDEL

SEQ ID NO: 15 - DNA, 40 bp, synthetic construct
  misc_feature 1..40: note = primer 9
  source 1..40: mol_type = other DNA
actaattattcgaaacgaggatgcaattcaactggaatat

SEQ ID NO: 16 - DNA, 40 bp, synthetic construct
  misc_feature 1..40: note = primer 10
  source 1..40: mol_type = other DNA
acggccggctgggccacgtggtgataataattgctgttga

SEQ ID NO: 17 - DNA, 1548 bp, synthetic construct
  misc_feature 1..1548: note = Ogataea angusta PDI_nt sequence
  source 1..1548: mol_type = other DNA
atgaagctgtttaacgtaagtatattgacttctgtgttagctgtcatggccgtggcacgtggagacgccgatgaagcagcaattgcaagtcccgattcagcagtggtcaagctgacggcagagtcctttgagtcctttattaaagaaaatccccttgtccttgctgagttctttgcaccctggtgcggtcattgtaaaaggttaggcccagagttcagtgcagcagctgataaattggtggagaaggatataaagttagcacaaatagactgcacccaggaaagggatttatgtgcagactacggcattaggggttacccctcactgaaggtgtttagaggtaacaattcaccaagtgactatcagggacaacgtgaacaggacgcaatagtaagttatatgattaaacaggctctgccacctgtctcccttttggaggatacagctgatttattggatgcactggccgaattatcagagccaatgatcttgcaagtattgccccccgattctaaatcatcaggaaatgagacgtttcactctttagccaatcgtctgcgtgatgagttccgtttcgtctcaacttccaatccagaatacgtggaaaaatatgttaaagagaaatccactccaacctacgtagtgttcaggcccggagagaaaacggaagatgcctccgttctaacaaacaagactatagacgaagagggcctggagaaatttatcagtgtggagaccaagcctctatttggagaggtgaccggagccacttttcaatcatacatggattctaagatacctttagcatatttcttttacgaagaggagtctcagaaagctgcagtggcagatgagattacaaagttagccaaaaagtacagaggtgagattaatttcgcaggcttagaggctaagaaatatggactgcacgccaagaatttgaatatgcaggaaaaattcccattgttcgctatacacgacctacagggtgacttaaagtatggaataagtcaggacaaggacctagacttctccgaaatcccaaagtttgtagaaaacttcaaaaaaggaaaattagagcccatagtaaaatctgagccaattcctgaaactcaagaagaagctgtctaccatctggtcggctatgagcatgataagattgtcaaccaagaaaaagatgtgttagtggaatactatgctccatggtgcggtcattgcaaaaggcttgctccaacttacgaggagttggctgctatctataaaaatgacaccgccgcttcagcaaaggtgttaatcgccaaaattgatcacaccgctaatgacgtcagtggtgtagaaataaccggctaccctacgatctttctttaccctgccgacggtagtggtcccgtaaactatgagggacagcgtaccctagaaagtttggccagtttcatccaagaaaagggcacgtttggagtagatggtctagcaatccgtgacgccaagtcagctggtgcagatggacccgaaagtgacgcaaaagactctacacacgacgaactgtaa

SEQ ID NO: 18 - DNA, 1509 bp, synthetic construct
  misc_feature 1..1509: note = Trichoderma reesei PDI_nt sequence
  source 1..1509: mol_type = other DNA
atgcaacagaagcgtcttactgctgccctggtggccgctttggccgctgtggtctctgccgagtcggatgtcaagtccttgaccaaggacaccttcaacgacttcatcaactccaatgacctcgtcctggctgagttcttcgctccctggtgcggccactgcaaggctctcgcccccgagtacgaggaggcggccacgactctcaaggacaagagcatcaagctcgccaaggtcgactgtgtcgaggaggctgacctctgcaaggagcatggagttgagggctaccccacgctcaaggtcttccgtggcctcgataaggtcgctccctacactggtccccgcaaggctgacggcatcacctcctacatggtgaagcagtccctgcctgccgtctccgccctcaccaaggataccctcgaggacttcaagaccgccgacaaggtcgtcctggtcgcctacatcgccgccgatgacaaggcctccaacgagaccttcactgctctggccaacgagctgcgtgacacctacctctttggtggcgtcaacgatgctgccgttgctgaggctgagggcgtcaagttcccttccattgtcctctacaagtccttcgacgagggcaagaacgtcttcagcgagaagttcgatgctgaggccattcgcaactttgctcaggttgccgccactcccctcgttggcgaagttggccctgagacctacgccggctacatgtctgccggtatccctctggcttacatcttcgccgagaccgccgaggagcgtgagaacctggccaagaccctcaagcccgtcgccgagaagtacaagggcaagatcaacttcgccaccatcgacgccaagaactttggctcgcacgccggcaacatcaacctcaagaccgacaagttccccgcctttgccattcacgacattgagaagaacctcaagttcccctttgaccagtccaaggagatcaccgagaaggacattgccgcctttgtcgacggcttctcctctggcaagattgaggccagcatcaagtccgagcccatccccgagacccaggagggccccgtcaccgttgtcgttgcccactcttacaaggacattgtccttgacgacaagaaggacgtcctgattgagttctacgctccctggtgcggtcactgcaaggctctcgcccccaagtacgatgagctcgccagcctgtatgccaagagcgacttcaaggacaaggttgtcatcgccaaggttgatgccactgccaacgacgtccccgacgagatccagggcttccccaccatcaagctctaccccgccggtgacaagaagaaccccgtcacctacagcggtgcccgcactgttgaggacttcatcgagttcatcaaggagaacggcaagtacaaggccggcgtcgagatccccgccgagcccaccgaggaggctgaggcttccgagtccaaggcctctgaggaggccaaggcttccgaggagactcacgatgagctgtaa

SEQ ID NO: 19 - DNA, 20 bp, synthetic construct
  misc_feature 1..20: note = primer 11
  source 1..20: mol_type = other DNA
actaattattcgaaacgagg

SEQ ID NO: 20 - DNA, 20 bp, synthetic construct
  misc_feature 1..20: note = primer 12
  source 1..20: mol_type = other DNA
acggccggctgggccacgtg

SEQ ID NO: 21 - DNA, 22 bp, synthetic construct
  misc_feature 1..22: note = primer 13
  source 1..22: mol_type = other DNA
gtaaaaaaggagtagaaacatt

SEQ ID NO: 22 - DNA, 40 bp, synthetic construct; identical to SEQ ID NO: 8
  misc_feature 1..40: note = primer 14
  source 1..40: mol_type = other DNA

SEQ ID NO: 23 - DNA, 40 bp, synthetic construct
  misc_feature 1..40: note = primer 15
  source 1..40: mol_type = other DNA
agaaagtataggaacttcgcggatccgcacaaacgaaggt

SEQ ID NO: 24 - protein, 583 aa, synthetic construct
  REGION 1..583: note = Bovine albumin_amino acid sequence
DTHKSEIAHRFKDLGEEHFKGLVLIAFSQYLQQCPFDEHVKLVNELTEFAKTCVADESHAGCEKSLHTLFGDELCKVASLRETYGDMADCCEKQEPERNECFLSHKDDSPDLPKLKPDPNTLCDEFKADEKKFWGKYLYEIARRHPYFYAPELLYYANKYNGVFQECCQAEDKGACLLPKIETMREKVLASSARQRLRCASIQKFGERALKAWSVARLSQKFPKAEFVEVTKLVTDLTKVHKECCHGDLLECADDRADLAKYICDNQDTISSKLKECCDKPLLEKSHCIAEVEKDAIPENLPPLTADFAEDKDVCKNYQEAKDAFLGSFLYEYSRRHPEYAVSVLLRLAKEYEATLEECCAKDDPHACYSTVFDKLKHLVDEPQNLIKQNCDQFEKLGEYGFQNALIVRYTRKVPQVSTPTLVEVSRSLGKVGTRCCTKPESERMPCTEDYLSLILNRLCVLHEKTPVSEKVTKCCTESLVNRRPCFSALTPDETYVPKAFDEKLFTFHADICTLPDTEKQIKKQTALVELLKHKPKATEEQLKTVMENFVAFVDKCCAADDKEACFAVEGPKLVVSTQTALA

SEQ ID NO: 25 - DNA, 1752 bp, synthetic construct
  misc_feature 1..1752: note = Bovine albumin_nt sequence
  source 1..1752: mol_type = other DNA
gatacccataagtcagagatcgcccaccgtttcaaggacttaggcgaagagcatttcaagggattggtactaatagcattttcacaatacctgcagcagtgcccttttgatgagcatgtgaaattagtgaacgagctgacagagttcgctaagacgtgcgtggcagatgaatcccatgcaggctgtgaaaaatcactgcatacactattcggagacgaattatgtaaggtcgccagtttaagagaaacatatggcgacatggctgattgttgcgagaaacaagaacccgagagaaatgaatgttttttgtcccacaaggacgattcccctgacttgccaaaactgaagcctgaccccaatacattgtgtgatgagtttaaggccgatgagaagaagttctggggcaagtacttgtatgaaatagcaaggaggcacccttatttctatgcaccagaattactatattacgcaaataagtacaacggtgttttccaagaatgctgccaggccgaggataaaggagcatgccttctgcctaagatagaaacgatgcgtgaaaaggtgttggcatctagtgcaagacaacgtctaaggtgcgcctctattcaaaagttcggcgaaagggctttgaaagcttggtctgtggcacgtctgtcacagaagttcccaaaggccgaattcgtggaagtcacaaaactagttactgacttaacaaaagtgcacaaggagtgttgtcatggcgacctgcttgaatgtgctgacgatagagcagacctagcaaagtatatatgcgataaccaagacacgatctcctctaagttgaaggaatgttgtgataagccactactggagaagtcacattgtattgcagaagtcgagaaagatgcaattcccgagaacctgccacccttaactgctgattttgccgaggacaaagacgtgtgtaagaactaccaggaggccaaggacgcatttttgggatccttcctttatgagtactctcgtagacatcctgagtacgctgtttcagtcttgctgcgtttggctaaagagtacgaagctacccttgaagagtgctgcgcaaaagatgatccccatgcttgctactctactgtgttcgataagcttaaacatctggtggacgaaccccagaatctaattaagcagaactgcgatcagttcgaaaagctgggagagtatggatttcagaacgcactaatcgtaaggtatacgcgtaaagtcccacaagtatccactcccacgttggttgaagtctcaagaagtctaggtaaagttggaacgagatgttgtacgaagcccgaatccgaaaggatgccttgtactgaggattacttatccctgattttaaacaggctgtgcgtacttcacgagaagacgcccgtttccgagaaagttaccaagtgttgtacagaaagtctagttaacagaaggccttgtttcagtgcactgactcctgatgaaacttacgtgcccaaagctttcgatgagaaattatttacgtttcatgccgacatatgcacgctgcccgatactgaaaaacaaataaagaaacagaccgcattggttgaactactgaaacacaagcccaaggctaccgaagaacaacttaagacggttatggaaaactttgtagccttcgtggacaaatgttgcgctgctgatgacaaggaggcatgcttcgctgtggagggacccaaactagtcgtatcaactcagaccgcactggcctaa

SEQ ID NO: 26 - DNA, 20 bp, synthetic construct
  misc_feature 1..20: note = primer 16
  source 1..20: mol_type = other DNA
gggtatctctcgagaaaaga

SEQ ID NO: 27 - DNA, 20 bp, synthetic construct
  misc_feature 1..20: note = primer 17
  source 1..20: mol_type = other DNA
tcatgtctaaggctacaaac

SEQ ID NO: 28 - DNA, 20 bp, synthetic construct
  misc_feature 1..20: note = primer 18
  source 1..20: mol_type = other DNA
gtttgtagccttagacatga

SEQ ID NO: 29 - DNA, 20 bp, synthetic construct
  misc_feature 1..20: note = primer 19
  source 1..20: mol_type = other DNA
tcttttctcgagagataccc

SEQ ID NO: 30 - protein, 57 aa, synthetic construct
  REGION 1..57: note = Bovine insulin precursor_amino acid sequence
EPKFVNQHLCGSHLVEALYLVCGERGFFYTPKAAAKGIVEQCCASVCSLYQLENYCN

SEQ ID NO: 31 - DNA, 174 bp, synthetic construct
  misc_feature 1..174: note = Bovine insulin precursor_nt sequence
  source 1..174: mol_type = other DNA
gaaccaaaatttgttaatcaacacttatgtggttcccacttagtggaagccctttatctagtgtgcggagagcgtggctttttctatacccctaaggctgcagcaaagggtatcgtggagcaatgttgcgcctctgtatgcagtctttaccaacttgaaaattactgcaattaa